European Patent Specification EP 3 808 357 B1, published March 26, 2025. Title: Composition and use thereof. Applicant: BGI SHENZHEN. The sequence listing filed with the application follows.

SEQUENCE LISTING (7 sequences)

SEQ ID NO: 1 - DNA, 20 bp, Artificial Sequence
  synthetic primer
agagtttgatcatggctcag

SEQ ID NO: 2 - DNA, 22 bp, Artificial Sequence
  synthetic primer
tagggttaccttgttacgactt

SEQ ID NO: 3 - DNA, 1423 bp, Artificial Sequence
  Megamonas funiformis AF24-28AC 16S rDNA
ttaacacatgcaagtcgaacggggtgtttatttcggtaaacaccaagtggcgaacgggtgagtaacgcgtaagcaatctaccttcaagatggggacaacacttcgaaaggggtgctaataccgaatgaatgtaagagtatcgcatgagacacttactaaaggaggcctctgaaaatgcttccgcttgaagatgagcttgcgtctgattagctagttggtgagggtaaaggcccaccaaggcgacgatcagtagccggtctgagaggatgaacggccacattgggactgagacacggcccagactcctacgggaggcagcagtggggaatcttccgcaatgggcgaaagcctgacggagcaacgccgcgtgaacgatgaaggtcttaggatcgtaaagttctgttgttagggacgaagggtaagaataataatacggtttttatttgacggtacctaacgaggaagccacggctaactacgtgccagcagccgcggtaatacgtaggcggcaagcgttgtccggaattattgggcgtaaagggagcgcaggcgggaaactaagcggatcttaaaagtgcggggctcaaccccgtgatggggtccgaactggttttcttgagtgcaggagaggaaagcggaattcccagtgtagcggtgaaatgcgtagatattgggaagaacaccagtggcgaaggcggctttctggactgtaactgacgctgaggctcgaaagctagggtagcgaacgggattagataccccggtagtcctagccgtaaacgatggatactaggtgtgggaggtatcgaccccttccgtgccggagttaacgcaataagtatcccgcctggggagtacggccgcaaggttgaaactcaaaggaattgacgggggcccgcacaagcggtggagtatgtggtttaattcgacgcaacgcgaagaaccttaccaagacttgacattgattgaaaggcctagagataggtcccttctcttcggagaacaagaaaacaggtggtgcatggctgtcgtcagctcgtgtcgtgagatgttgggttaagtcccgcaacgagcgcaacccctatactatgttgccagcattacggatgggaactcatagtagactgccgcggacaacgcggaggaaggcggggatgacgtcaagtcatcatgccccttacgtcttgggctacacacgtactacaatgggatgaacagagggaagcgaaatcgcgaggtggagcggatccctaaaagcatctctcagttcggattgtaggctgaaactcgcctacatgaagtcggaatcgctagtaatcgcaggtcagcatactgcggtgaatacgttcccgggccttgtacacaccgcccgtcacaccacgaaagtcattcacacccgaagccggctaagggcctatggtac

SEQ ID NO: 4 - DNA, 1425 bp, Artificial Sequence
  Anaerofustis stercorihominis AM25-6 16S rDNA
acgaacgctggcggcgtgcttaacacatgcaagtcgaacgagaagcttataaatgatccttcgggtgaagctataagcggacagtggcgaacgggtgagtaacgcgtaggtaaccaacctcatgcagggggatagcccagggaaacttggattaaacccgcataagaccacagcaccgcatggtgcaggggtaaaaactccggtggcatgagacggacctgcgtcttattaggtagttggtgaggtaacggctcaccaagccaacgatgagtagccgacctgagagggtgatcggccacattgggactgagacacggcccagactcctacgggaggcagcagtggggaatattgcgcaatgggggaaaccctgacgcagcaacgccgcgtgagcgatgaaggttttcggatcgtaaagctctgtctttggggaagataatgacggtacccaaggaggaagctccggctaactacgtgccagcagccgcggtaatacgtagggagcaagcgttgtccggattcactgggcgtaaagagcacgtaggcggttaattaagtcaggtgtgaaagttttcggctcaaccggaaaagtgcacttgaaactggataacttgagtatcggagaggtaagcggaattcctagtgtagcggtgaaatgcgtagagattaggaagaacaccggtggcgaaggcggcttactggacgataactgacgctgaggtgcgaaagcgtggggagcgaacaggattagataccctggtagtccacgccgtaaacgatgaatactaggtgttggggtaactcagtgccgcagttaacacattaagtattccgcctggggagtacgctcgcaagagtgaaactcaaaggaattgacgggggcccgcacaagcagcggagcatgtggtttaattcgaagcaacgcgaagaaccttaccaggtcttgacatcccttgaccgcctaagagattaggctttccttcgggacaaggagacaggtggtgcatggttgtcgtcagctcgtgtcgtgagatgttgggttaagtcccgcaacgagcgcaacccttatgtttagttactaacattcagttgaggactctagacagactgcccttgaaagagggaggaaggtggggacgacgtcaaatcatcatgccccttacgacctgggctacacacgtgctacaatggtctgtacagagggttgcgaagcagtgatgctaagctaatctcaaaaagcagatctcagttcggattgcaggctgcaactcgcctgcatgaagtcggagttgctagtaatcgcgaatcagaatgtcgcggtgaatgcgttcccgggccttgtacacaccgcccgtcacaccacgagagttggtaacacccgaagccagtgagctaaccattaggaggcagctgtcgaaggtggga

SEQ ID NO: 5 - DNA, 1380 bp, Artificial Sequence
  Collinsella shenzhenensis TF06-26 16S rDNA
cggcacccctctccggagggaagcgagtggcgaacggctgagtaacacgtggagaacctgccccctcccccgggatagccgcccgaaaggacgggtaataccggataccccggggtgccgcatggcaccccggctaaagccccgacgggaggggatggctccgcggcccatcaggtagacggcggggtgacggcccaccgtgccgacaacgggtagccgggttgagagaccgaccggccagattgggactgagacacggcccagactcctacgggaggcagcagtggggaatcttgcgcaatggggggaaccctgacgcagcgacgccgcgtgcgggacggaggccttcgggtcgtaaaccgctttcagcagggaagagtcaagactgtacctgcagaagaagccccggctaactacgtgccagcagccgcggtaatacgtagggggcgagcgttatccggattcattgggcgtaaagcgcgcgtaggcggcccggcaggccgggggtcgaagcggggggctcaaccccccgaagcccccggaacctccgcggcttgggtccggtaggggagggtggaacacccggtgtagcggtggaatgcgcagatatcgggtggaacaccggtggcgaaggcggccctctgggccgagaccgacgctgaggcgcgaaagctgggggagcgaacaggattagataccctggtagtcccagccgtaaacgatggacgctaggtgtggggggacgatccccccgtgccgcagccaacgcattaagcgtcccgcctggggagtacggccgcaaggctaaaactcaaaggaattgacgggggcccgcacaagcagcggagcatgtggcttaattcgaagcaacgcgaagaaccttaccagggcttgacatatgggtgaagcgggggagaccccgtggccgagaggagcccatacaggtggtgcatggctgtcgtcagctcgtgtcgtgagatgttgggttaagtcccgcaacgagcgcaacccccgccgcgtgttgccatcgggtgatgccgggaacccacgcgggaccgccgccgtcaaggcggaggagggcggggacgacgtcaagtcatcatgccccttatgccctgggctgcacacgtgctacaatggccggtacagagggatgccaccccgcgagggggagcggatcccggaaagccggccccagttcggattgggggctgcaacccgcccccatgaagtcggagttgctagtaatcgcggatcagcatgccgcggtgaatgcgttcccgggccttgtacacaccgcccgtcacaccacccgagtcgtctgcacccgaagtcgccggcccaaccgagaggggggaggcgccgaaggtgtggagggtg

SEQ ID NO: 6 - DNA, 1400 bp, Artificial Sequence
  Lactobacillus gasseri TF08-1 16S rDNA
ggtgcttgcaccagatgaaactagatacaagcgagcggcggacgggtgagtaacacgtgggtaacctgcccaagagactgggataacacctggaaacagatgctaataccggataacaacactagacgcatgtctagagtttaaaagatggttctgctatcactcttggatggacctgcggtgcattagctagttggtaaggtaacggcttaccaaggcaatgatgcatagccgagttgagagactgatcggccacattgggactgagacacggcccaaactcctacgggaggcagcagtagggaatcttccacaatggacgcaagtctgatggagcaacgccgcgtgagtgaagaagggtttcggctcgtaaagctctgttggtagtgaagaaagatagaggtagtaactggcctttatttgacggtaattacttagaaagtcacggctaactacgtgccagcagccgcggtaatacgtaggtggcaagcgttgtccggatttattgggcgtaaagcgagtgcaggcggttcaataagtctgatgtgaaagccttcggctcaaccggagaattgcatcagaaactgttgaacttgagtgcagaagaggagagtggaactccatgtgtagcggtggaatgcgtagatatatggaagaacaccagtggcgaaggcggctctctggtctgcaactgacgctgaggctcgaaagcatgggtagcgaacaggattagataccctggtagtccatgccgtaaacgatgagtgctaagtgttgggaggtttccgcctctcagtgctgcagctaacgcattaagcactccgcctggggagtacgaccgcaaggttgaaactcaaaggaattgacgggggcccgcacaagcggtggagcatgtggtttaattcgaagcaacgcgaagaaccttaccaggtcttgacatccagtgcaaacctaagagattaggtgttcccttcggggacgctgagacaggtggtgcatggctgtcgtcagctcgtgtcgtgagatgttgggttaagtcccgcaacgagcgcaacccttgtcattagttgccatcattaagttgggcactctaatgagactgccggtgacaaaccggaggaaggtggggatgacgtcaagtcatcatgccccttatgacctgggctacacacgtgctacaatggacggtacaacgagaagcgaacctgcgaaggcaagcggatctctgaaagccgttctcagttcggactgtaggctgcaactcgcctacacgaagctggaatcgctagtaatcgcggatcagcacgccgcggtgaatacgttcccgggccttgtacacaccgcccgtcacaccatgagagtctgtaacacccaaagccggtgggataacctttatagga

SEQ ID NO: 7 - DNA, 1380 bp, Artificial Sequence
  Lactobacillus acidophilus AM13-1 16S rDNA
tgcctaatacatgcaagtcgagcgagctgaaccaacagattcacttcggtgatgacgttgggaacgcgagcggcggatgggtgagtaacacgtggggaacctgccccatagtctgggataccacttggaaacaggtgctaataccggataagaaagcagatcgcatgatcagcttataaaaggcggcgtaagctgtcgctatgggatggccccgcggtgcattagctagttggtagggtaacggcctaccaaggcaatgatgcatagccgagttgagagactgatcggccacattgggactgagacacggcccaaactcctacgggaggcagcagtagggaatcttccacaatggacgaaagtctgatggagcaacgccgcgtgagtgaagaaggttttcggatcgtaaagctctgttgttggtgaagaaggatagaggtagtaactggcctttatttgacggtaatcaaccagaaagtcacggctaactacgtgccagcagccgcggtaatacgtaggtggcaagcgttgtccggatttattgggcgtaaagcgagcgcaggcggaagaataagtctgatgtgaaagccctcggcttaaccgaggaactgcatcggaaactgtttttcttgagtgcagaagaggagagtggaactccatgtgtagcggtggaatgcgtagatatatggaagaacaccagtggcgaaggcggctctctggtctgcaactgacgctgaggctcgaaagcatgggtagcgaacaggattagataccctggtagtccatgccgtaaacgatgagtgctaagtgttgggaggtttccgcctctcagtgctgcagctaacgcattaagcactccgcctggggagtacgaccgcaaggttgaaactcaaaggaattgacgggggcccgcacaagcggtggagcatgtggtttaattcgaagcaacgcgaagaaccttaccaggtcttgacatctagtgcaatccgtagagatacggagttcccttcggggacactaagacaggtggtgcatggctgtcgtcagctcgtgtcgtgagatgttgggttaagtcccgcaacgagcgcaacccttgtcattagttgccagcattaagttgggcactctaatgagactgccggtgacaaaccggaggaaggtggggatgacgtcaagtcatcatgccccttatgacctgggctacacacgtgctacaatggacagtacaacgaggagcaagcctgcgaaggcaagcgaatctcttaaagctgttctcagttcggactgcagtctgcaactcgactgcacgaagctggaatcgctagtaatcgcggatcagcacgccgcggtgaatacgttcccgggccttgtacacaccgc